European Patent Application EP 4 772 526 A1, published July 8, 2026. Title: Novel Peptide Having Activity of Improving Skin Condition and Uses Thereof. Applicant: CAREGEN CO., LTD. Application KR. The sequence listing filed with the application follows.

SEQUENCE LISTING (13 sequences)

SEQ ID NO: 1 - protein, 8 aa, synthetic construct
DRKKIQNK

SEQ ID NO: 2 - DNA, 20 bp, synthetic construct
  source 1..20: mol_type = other DNA
caccctcaagagcctgagtc

SEQ ID NO: 3 - DNA, 20 bp, synthetic construct
  source 1..20: mol_type = other DNA
agacggctgagtagggaaca

SEQ ID NO: 4 - DNA, 20 bp, synthetic construct
  source 1..20: mol_type = other DNA
ccaggaaccgagtacaccat

SEQ ID NO: 5 - DNA, 20 bp, synthetic construct
  source 1..20: mol_type = other DNA
atacccaggttgggtgatga

SEQ ID NO: 6 - DNA, 20 bp, synthetic construct
  source 1..20: mol_type = other DNA
gcaagacctggctttggact

SEQ ID NO: 7 - DNA, 21 bp, synthetic construct
  source 1..21: mol_type = other DNA
gggagtttctggttagggctg

SEQ ID NO: 8 - DNA, 20 bp, synthetic construct
  source 1..20: mol_type = other DNA
ccttcttgggtgctggaata

SEQ ID NO: 9 - DNA, 20 bp, synthetic construct
  source 1..20: mol_type = other DNA
acacgataagggaggctgtg

SEQ ID NO: 10 - DNA, 20 bp, synthetic construct
  source 1..20: mol_type = other DNA
tcagtggctggaacagtgag

SEQ ID NO: 11 - DNA, 20 bp, synthetic construct
  source 1..20: mol_type = other DNA
tctggcatgtcccactatca

SEQ ID NO: 12 - DNA, 20 bp, synthetic construct
  source 1..20: mol_type = other DNA
ggagccaaaagggtcatcat

SEQ ID NO: 13 - DNA, 20 bp, synthetic construct
  source 1..20: mol_type = other DNA
gtgatggcatggactgtggt